European Patent Application EP 4 644 536 A1, published November 5, 2025. Title: 干细胞及其制备方法和应用、及治疗骨缺损的方法. Applicant: 西北工业大学. Application CN. The sequence listing filed with the application follows.

SEQUENCE LISTING (9 sequences)

SEQ ID NO: 1 - DNA, 1000 bp, Cervus nippon
  source 1..1000: mol_type = genomic DNA
atgggtgcccagttctccaagaccgccgcgaagggagaagccaccacggagaggcccggggaggcggctgtggcctcgtcgccttctaaagcgaatgggcaggaaaatggccacgtgaaggtaaacggcgacgcttctcccgcggccgccgagcccggcgccaaggaggagctgcaggccaacggcagcgccccggctgccgacaaggaggagcccgcggccgccgggagcggggcggcgtcgcccgccgcggccgagaaggatgagccggccgctgctgcccccgacgccggggccagccccgcggagaaggaagcccccgtggagggcgaggccgccgagcccggctcacccacggccgccgagggggaggccgcctctgccgcctcctcgacgtcttcgccgaaggctgaggacggggccacgccctcgcccagcaacgagaccccgaaaaaaaaaaagaagcgcttttccttcaagaagtctttcaagctgagcggcttctccttcaagaagaacaagaaggaggcaggagagggcggtgaggccgaaggggccgccggcgcctccgccgaaggcggcaaggacgaggcctctgggggcgccgctgcggccgccggcgaggcgggtgcggccccgggagccggcagcggcgcggggcgaggaggcggccgcgggcgaggagggggcggcggggggcgacccgcaggaggccaagcccgaggaggctgccgtcgcgcccgagaagccgcccgccagcgaggaggcgaaggcagtcgaggagcccagcaaggccgaggagaaggcagaagaggccggggccagcgcggccggctgcgaggcgccctcggccgccgggcccggcgtgcccccagagcaggaggcggcccccgcggaggaggcggcggccgccccggcgtcgtcagcctgcgcagccccctcacaggaggcccagcccgagtgcagtccagaagcgcccccagcggaggcagccgagtaa

SEQ ID NO: 2 - DNA, 888 bp, Cervus nippon
  source 1..888: mol_type = genomic DNA
atgctagatgtgactcagccgctcactgtgggacccaacgaacggctaaccgacaggtcggagtctcaccctcgggatcttaaaaggccgggagagctcccgtggcctcctccctccaggaggtggggactaggtggaggaagggctgcgggaggaggagctggcgcgtcgcgacccgccccgtcccatccagtctggcctgggcgccgaaggaactgcggtcctagcccctgtcatccagcggcttgtcctgcgtgccccgagccctgcccgcacccagttatgactctgcgcccctcacttctcccgctccgactgctgctgctgctgctgctcaggggggcggtgtgccgggcggaggctgggtccgaaaccgaaagtcccgtccggaccctccaagtggagaccctggtggagccccccgagccgtgtgctgagcctgctgcctttggagacacgcttcacatacactactcgggcagcctggtagatggacgcatctttgacacgtctctgagcagagaccctctggttatagaacttggccaaaagcaggtgataccaggtctggagcagagccttctagacatgtgtgtgggagagaagcgaagggtaatcattccttctcacctggcctatggaaaacggggatttccaccatctatcccagcggatgcagagctgcattttgacgtggaactgattgcactgatccgagccaactactggcagaagctggtgaagggcattttgcctctggtaggcatggccatggtgccagccctcctgggccttattggctatcatctatacagaaaggccagcagtcctaaaatctccaaaaagaagctcaaggaagagaaacgaaacaagagcaaaaagaaataa

SEQ ID NO: 3 - DNA, 654 bp, Cervus nippon
  source 1..654: mol_type = genomic DNA
atgggctacagcccaccaggctcctctgtccgtaaattttccaggcaagaatactggaaacctcagcctgctgccttctttgcaattatccaaaatatccttgaagtggctgtttacacaacattaaaatggggagcaaggccacaaatgcagactccacagtacctgcagcaacgtcgaaaatttgcagctgccttcttggcatttattttcatcttggcagttgtggacacggctgaagcaggaaagaaagagaaaccagagaagaaggtgaagaagtctgactgtggagagtggcagtggagtgtgtgtgtgcccaccagcggggactgtgggctgggcacccgcgagggcacccgcacgggagccgagtgtaaacagaccatgaagacccagaggtgtaagatcccctgcaactggaaaaagcagtttggagcggagtgcaaataccagttccaggcctggggagaatgtgatctgaacacggctctgaagaccagaactgggagcctgaagcgagccctccacaacgccgactgccagaagacagtcaccatctccaagccctgtggcaagctgactaagtccaaacctcaagcagaatctaagaagaagaaaaaggaaggcaagaaacaggagaagatgctggactaa

SEQ ID NO: 4 - DNA, 4515 bp, Cervus nippon
  source 1..4515: mol_type = genomic DNA
atgctctcaattctaagaagcaaaatcctgactcaagaaagtgctgaagtagaaaacttgcatgctatgttgcatctggctctttccgaccccacggatgatagcccccaggcttctctgcccatgggattttccaggcaagaatactggagtgggttgccatttccttctccaggggatcttccagattcagggactgagccagtgtctcttgcatctcttgcattggcaggggatcttcctgacccaggaagtgaacccacatctcctgctttggcaggagaattctttatgattgagccaccagggaaggccttgtgtatcacaggcttccaggagcatcggttccctgtctccccaaggatgggtctccaggggaggttctgcttccccctggggctcctgttgggctatgtgctcttggtggcctcggccccagccactctcgagtcttctggatgcagcgagaaggagcagcaggtcactgtcagccacacctacaagatcgacgtgcccaagtccgccttggtccaggtggaggctgacccccagccccttcgtggtgatggaacctcgctcctggccccagaggagatcgaggaacagaatatcgtcttcaggcacaacatccgcctgcagacgccacaggactgtgagctggcaggcagcgtgcgggacctcctggcccgggtgaagaagctggaggaggagatggcggaggtgaaggagcggtgcagcgccgagcgctgctgcgcgggagcagctggtctgagccgccactgcagcggccacgggaccttctccctggacacgtgcagctgccactgcgagcatggctgggagggcgccgactgcgagcggctcgcctgccccggcgcctgcagcggccacgggcgctgcgtgaacggcagctgcgtgtgcgagccgccctacgtgggcgccgactgcgcctaccccgcctgccccgagaactgcagcgggcacggcacatgcgtgcgtggcgtctgccagtgccacgaggacttcacgtcggaggactgcagcgagcggcgctgccccggcgactgcagcggccacggcttctgcgacaccggcgagtgttactgcgaggagggcttcaccggcctcgactgcgcccgggtggttgccccccagggactgcagctgctcaagagcacagaggattccctgctggtcagctgggagcccaccagccaggtggaccactacctcctcagctactacccactggggaaggagctctccgtgaagcatgtcagagtgcccaaggagcagcacagctacgagatccttggtttgctgcctggaaccaagtacatcgtgaccctgcgcaatgtgaagaaagagatttccagtagcccacagcatctactggccaccacagatcttgctgtgcctggcactgcctgggtgacggatgagacggagaactcccttgacgtggaatgggagaaccccccgaccgaggtggactattacaagttgcagtatggcccactgacagggcacgaggtggccgaggtcaccgtgcccaagagcggtgaccccaagagccaatacgacatcacaggtctgcagccggggacggaatataagatcgcagtcatccctatgaggggagacctcgagggcaagccgattcttctgaacggcaggacagatatcgatagtccaaccaacgtggtcactggccgagtgacagaagacacagtggcggtctcctgggacccagtccgggcggtcattgataagtacatggtgcgctacatctccgctgacggggagacgaaggacaccgcggtgcccggggagcagaacagcactgtcctgacaggtctgaagccgggggaggcctatgaagtctacgtgtgggctgagaggggcagccaggagagcaagaaggcggacaccacggccctcacagaaattgacagcccccagaacctggtgactaatcaggtgacggagaacacggccaccgtctcctgggacccggtgcaggctgacatcgacaggtacctggtgcgctacacctctgctgatggagacagcagggaggttctggtggggaaggagcagaccagcaccgtcctgatgggcctgaggccaggcgtggagtacacagtccacgtgtgggctgagaaggggaaccgggagagcaggaaggctgacaccaaggccccaacagaaattgacagcccccaaaacctggtgaccgagcaggtgacggagaacacggccaccgtctcctgggacccggtgcaggccgtcatcgacaggtacctggtgcgctacacctctgctgacggagacagcagggaggttccggtagggaaggagcagagcagcactgtcctgacgggcctgaggccaggcgtggagtacacggtccacgtgtgggcccagaagggggaccaggagagcaggaaggccgacaccaaggcccctacagacattgacagccccaaaaacctggtgactgagcaggtgacggagaacacggccaccgtctcctgggacccggtgcaggccgtcatcgacaggtacctggtgagctacacctctgctgatggagacaccagagaggttccggtggggaaggagcagagcagcaccgtcctgacgggcctgaggccaggcgtggagtacacagtccacgtgtgggcccagaagggggaccaggagagcaggaaggctgacaccaaggccccgacagacattgacagcccccaaaacctggtgaccgagcaggtgacagagaacacggccaccgtctcctgggacccggtgcaggccgtcatcgacaggtacctggtgcgctacacctctgctgacggagacgccagggagattccggtggggaaggagcagagcagcaccatcctgacgggcctgaggccaggcgtggagtacacggtccacgtgtgggcccagaagggggaccgggagagcaggaaggccgacaccaaggcccctacagacattgacagccccaaaaacctggtgaccaagcaggtgacagagaacacggccaccgtctcctgggacccggtgcaggccgtcatcgacaggtacctggtgcgctacacctctgctgacggagacaccagagaggttccggtggggaaggagcagagcagcaccgtcctgacgggtctgaggccaggcgtggagtacacagtccatgtgtgggcccagaaggaggaccgggagagcaggaaggccgacactaaggccgctacagaaattgacagccccaaaaacctggtgaacgatcaggtgacggagaacacggccaccgtctcctgggacccggtgcaggccgtcatcgacaggtacctggtgcgctacacctctgctgacggagacaccagagaggttccggtggggaaggagcagagcagcaccgtcctgacgggcctgaggccaggtgtggagtacacggtccacgtgtgggcccagaaggaggaccgggagagcaggaaggccgacaccaaggccctgacagacattgaccctccccaaaaccttcgtccttctgctgtaacccagtctggtggggtattgacctggacacccccctctgccaacatcgatggctatattctgacctaccagttcccagacggcaccgtcaaggaggtgcagcttggaagaggggaccagaggtttgagttgcaaggccttgagcagggtgtcaccctccctatctccttagttgcctttaagggtgatcgccggagcaggagtgtatctaccaacctttccacagttggtgcccgttttccacacccttcggactgcagtcaggttcagcagaacagtaacgtcgccagtggcctctacaccatctacctgcacggggatgccagccggcccctgcaggtgtactgtgacatggacacagatggaggtggctggattgtcttccagaggcggaacactgggcaactggatttcttcaagcgctggcggacctacgtggaaggcttcggggaccccatgaaggagttctggcttggacttgacaagctacacaacctcaccatgggcacgcccacccgctatgaggtgagagtggacttacagactgccaatgaatctgcctatgccgtgtacgactccttccaggtggcctccagcaaggagcggtacaggctcacagtcgggaaatacagaggcacagcaggggacgcgctcagttaccacaacggatggaagtttacaacctttgaccgagacaacgacatcgccctcagcaactgtgccctgacgcatcacggcggctggtggtacaagaactgccacttggccaaccccaacggcagatacggggagaccaagcatagtgagggggtgaactgggagccatggaagggacatgaattctccattccttttgtggagttgaagatccgacctcacggctacagcggggagcatgttctgggcagaaagaaacgaatgctgggagaaaattcaagaacgttctaa

SEQ ID NO: 5 - DNA, 1269 bp, Cervus nippon
  source 1..1269: mol_type = genomic DNA
atgggcttttcaagtccagtatgtgtccttttcttctttcttggagtcaaagtatattgccaatatgaaagttatcaatgggatgaagattatgaccaagaaccagatgatgtctaccagacagaattccaatttcaacaaaatataaactatgaagctccatttcatcagcatactttaggttgtgccagtgaatgcttctgtccacctaactttccatcatcaatgtactgtgataatcgcaaattaaagactatcccaaatattccagcacacattcagcaagtctatcttcagttcaatgaaattgaggctgtgactgcagattcatttatcaatgccactcatcttaaagaaatcaacctcagccacaataaaattaaatctcaaaagattgatcatggtgtgtttgctaaattgtcaaatctactacagcttcacctacagcataacaatttagaagactttccatttcctcttcctaagtctttggaaaggatttttctaggttacaatgaaatttccagactgcagacaaatgctgtgaatgggcttgtaaacctgaccatgcttgatctctgttttaatcaaattgatgattctatgttacaagcaaaagtacttgccaaaatggaaaaattgatgcagctcaacctatgtaataacagattagaatcaatgcctcctggtttgccttcttcacttatgtatctgtctttagaaaacaattcaatatcttctataccagaaaattacttcaacgaacttccgaaacttcacgctctaagaatatcacacaacaaactacaagacattccatataatatttttaatctttccaaccttatagagctcaatgttggacacaacaaactgaagcaagcattctatattccaaggaatttagaacacctatacctagaaaataatgaaattgaaaatatcaatgtcacagtgatgtgtccatcagttgatccactacattaccaccatttaacatacattcgcgtagatcaaaataagctgaaagcgccaataagctcatacattttcctctgcttccctcatatacacactatttattatggtgaacaacaaagcactaatggtcaaacgatacaactgaagacccaagttttcaggagatttccagatgatggtgatagtgaagatcatgatgatcatcatgaaggcccagaagaagaagcaacagaagaaaacattgatgctaactattatggaagtcaagaatggcaaggaactgtatag

SEQ ID NO: 6 - DNA, 1167 bp, Cervus nippon
  source 1..1167: mol_type = genomic DNA
atggacggaccctgtgaagcagctccagccgagatgtgcgaggaggaggacagcaccgccctggtgtgtgacaatggctctgggctctgtaaggccggctttgcgggggatgatgctcccagggctgttttcccatccatcgtgggacgtcctcgacatcagggggtgatggtgggaatgggacagaaagacagctacgtgggcgatgaagcacagagcaaaagaggaatcctgaccctgaagtacccgatagagcatggcatcatcaccaactgggacgacatggagaagatctggcaccactctttctacaatgagcttcgtgttgcccctgaagagcatccaaccctgctcactgaggcacccctgaaccccaaggccaaccgggagaaaatgacccagattatgtttgagactttcaatgtcccagccatgtatgtggctattcaggcggtgctgtcgctctatgcctctggacgtacaactggcattgtgctggactctggagatggtgtcacccacaacgtgcccatctatgagggctacgccctgccccacgccatcatgcgtctggacctggctggccgagatctcaccgactacctcatgaagatcctgaccgagcgaggctattccttcgtgaccaccgctgagcgtgagattgtccgggacatcaaggagaaactgtgctacgtagccctggactttgagaatgagatggccactgccgcatcctcctcctccctcgagaagagctatgagctgcctgatgggcaggtgatcaccatcgggaatgagcgtttccgctgccctgagaccctgttccagccctcattcatcgggatggagtctgctggcatccatgagaccacgtacaacagcatcatgaagtgtgatattgatatcaggaaggacctctatgctaacaacgtcctctccgggggtaccaccatgtaccccggcattgctgatcgcatgcagaaagagatcacggccctggcccccagcaccatgaagatcaagatcatcgcccctcccgagcgcaaatactctgtctggattggtggctccatcctggcctccctgtccaccttccagcagatgtggatcagcaaacaggagtacgatgaggccgggccatccatcgtccaccgcaaatgtttctaa

SEQ ID NO: 7 - DNA, 4695 bp, Cervus nippon
  source 1..4695: mol_type = genomic DNA
atgggggccatgactcagctgttggcaggtgtctttcttgctttccttgccctcgctaccgaaggtggggtcctcaagaaagtcatccggcacaagcgacagagtggggtgaacgccaccctgccagaagagaaccagccagtggtgtttaaccacgtttacaacatcaagctgccagtgggatcccagtgttcggtggatctggagtcagccagtggggagaaagacctggcaccgccttcagagcccagcgaaagctttcaggagcacacagtggatggggaaaaccagattgtcttcacacatcgcatcaacatcccccgccgggcctgtggctgtgccgcagcccctgatgttaaggagctgctgagcagactggaggagctggagaacctggtgtcttccctgagggagcaatgtactgcaggagcaggctgctgtctccagcctgccacaggccgcttggacaccaggcccttctgtagcggtcggggcaacttcagcactgaaggatgtggctgtgtctgcgaacctggctggaaaggccccaactgctctgagcccgaatgtccaggcaactgtcaccttcgaggccggtgcattgatgggcagtgcatctgtgacgacggcttcacgggcgaggactgcagccagctggcttgccccagcgactgcaatgaccagggcaagtgcgtaaatggagtctgcatctgtttcgaaggctacgccggggctgactgcagccgtgaaatctgcccagtgccctgcagtgaggagcacggcacatgtgtagatggcttgtgtgtgtgccacgatggctttgcaggcgatgactgcaacaagcctctgtgtctcaacaattgctacaaccgtggacgatgcgtggagaatgagtgcgtgtgtgatgagggtttcacgggcgaagactgcagtgagctcatctgccccaatgactgcttcgaccggggccgctgcatcaatggcacctgctactgcgaagaaggcttcacaggtgaagactgcgggaaacccacctgcccacatgcctgccacacccagggccggtgtgaggaggggcagtgtgtatgtgatgagggctttgccggtgtggactgcagcgagaagaggtgtcctgctgactgtcacaatcgtggccgctgtgtagacgggcggtgtgagtgtgatgatggtttcactggagctgactgtggggagctcaagtgtcccaatggctgcagtggccatggccgctgtgtcaatgggcagtgtgtgtgtgatgagggctatactggggaggactgcagccagctacggtgccccaatgactgtcacagtcggggccgctgtgtcgagggcaaatgtgtatgtgagcaaggcttcaagggctatgactgcagtgacatgagctgccctaatgactgtcaccagcacggccgctgtgtgaatggcatgtgtgtttgtgatgacggctacacaggggaagactgccgggatcgccaatgccccagggactgcagcaacaggggcctctgtgtggacggacagtgcgtctgtgaggacggcttcaccggccctgactgtgcagaactctcctgtccaaatgactgccatggccagggtcgctgtgtgaatgggcagtgcgtgtgccatgaaggatttatgggcaaagactgcaaggagcaaagatgtcccagtgactgtcatggccagggccgctgcgtggacggccagtgcatctgccacgagggcttcacaggcctggactgtggccagcactcctgccccagtgactgcaacaacttaggacaatgcgtctcgggccgctgcatctgcaacgagggctacagcggagaagactgctcagaggtgtctcctcccaaagacctcgttgtgacagaagtgacggaagagacggtcaacctggcctgggacaatgagatgcgggtcacagagtaccttgtcgtgtacacgcccacccacgagggtggtctggaaatgcagttccgtgtgcctggggaccagacgtccaccatcatccaggagctggagcctggtgtggagtactttatccgtgtatttgccatcctggagaacaagaagagcattcctgtcagcgccagggtggccacgtacttacctgcacctgaaggcctgaaattcaagtccatcaaggagacatctgtggaagtggagtgggatcctctagacattgcttttgaaacctgggagatcatcttccggaatatgaataaagaagatgagggagagatcaccaaaagcctgaggaggccagagacctcttaccggcaaactggtctagctcctgggcaagagtatgagatatctctgcacatagtgaaaaacaatacccggggccctggcctgaagagggtgaccaccacacgcttggatgcccccagccagatcgaggtgaaagatgtcacagacaccactgccttgatcacctggttcaagcccctggctgagatcgatggcattgagctgacctacggcatcaaagacgtgccaggagaccgtaccaccatcgatctcacagaggacgagaaccagtactccatcgggaacctgaagcctgacactgagtacgaggtgtccctcatctcccgcagaggtgacatgtcaagcaacccagccaaagagaccttcacaacaggcctcgatgctcccaggaatcttcgacgtgtttcccagacagataacagcatcaccctggaatggaggaatggcaaggcagctattgacagttacagaattaagtatgcccccatctctggaggggaccacgctgaggttgatgttccaaagagccaacaagccacaaccaaaaccacactcacaggtctgaggccgggaactgaatatgggattggagtttctgctgtgaaggaagacaaggagagcaatccagcgaccatcaacgcagccacagagttggacacgcccaaggaccttcaggtttctgaaactgcagagaccagcctgaccctgctctggaagacaccgttggccaaatttgaccgctaccgcctcaattacagtctccccacaggccagtgggtgggagtgcagcttccaagaaacaccacttcctatgtcctgagaggcctggaaccaggacaggagtacaatgtcctcctgacagccgagaaaggcagacacaagagcaagcccgcacgtgtgaaggcatccactgccatgggctccccaaaggaagtcattttctcagacatcactgaaaattcggctactgtcagctggagggcacccacagcccaagtggagagcttccggattacctatgtgcccattacaggaggtacaccctccatggtaactgtggacggaaccaagactcagaccaggctggtgaaactcatacctggcgtggagtaccttgtcagcatcatcgccatgaagggctttgaggaaagtgaacctgtctcagggtcattcaccacagctctggatggcccatctggcctggtgacagccaacatcactgactcagaagccttggccaggtggcagccagccattgccactgtggacagttatgtcatctcctacacaggcgagaaagtgccagaaattacacgcacggtgtccgggaacacagtggagtatgctctgaccgacctcgagcctgccacggaatacacactgagaatctttgcagagaaagggccccagaagagctcaaccatcactgccaagttcacaacagacctcgattctccaagagacttgactgctactgaggttcagtcggaaactgccctccttacctggcgacccccccgggcatcagtcaccggttacctgctggtctatgaatcagtggatggcacagtcaaggaagtcattgtgggtccagataccacctcctacagcctggcagacctgagcccatccacccactacacagccaagatccaggcactcaatgggcccctgaggagcaatatgatccagaccatcttcaccacaattggactcctgtaccccttccccaaggactgctcccaagcaatgctgaatggagacacgacctctggcctctacaccatttatctgaatggtgataaggctgaggcgctggaagtcttctgtgacatgacctctgatgggggtggatggattgtgttcctgagacgcaaaaacggacgcgagaacttctaccaaaactggaaggcatatgctgctggatttggggaccgcagagaagaattctggcttgggctggacaacctgaacaaaatcacagcccaggggcagtacgagctccgggtggacctgcgggaccatggggagacagcctttgctgtctatgacaagttcagcgtgggagatgccaagactcgctacaagctgaaggtggaggggtacagtgggacagcaggtgactccatggcctaccacaatggcagatccttctccacctttgacaaggacacagattcagccatcaccaactgtgctctgtcctacaaaggggctttctggtacaggaactgtcaccgtgtcaacctgatggggagatatggggacaataaccacagtcagggcgttaactggttccactggaagggccacgaacactcaatccagtttgctgagatgaagctgagaccaagcaacttcagaaatcttgaaggcaggcgcaaacgggcataa

SEQ ID NO: 8 - DNA, 2517 bp, Cervus nippon
  source 1..2517: mol_type = genomic DNA
atgggattaacgtccacatggagatatggaagaggacaggggatcggcaccgtaaccatggtcagctggggtcgcttcctctgcctggttgtggtcaccatggcagccttgtccctggcccggccctccttcaatttagttgacgataccacggttgagccggaagagccaccaaccaaataccaaatctcccaaccagaagtttacgtggctgcgccccgggagtcgctagagttgcgctgcctgttgcgagatgccgccatgatcagttggactaaggatggggtacacttggggcccaacaataggacagtgcttattggggagtatttgcagataaaaggcgccacgcctagagactccggcctctatgcttgtactgctgctaggaacgtagacagtgagactgtctacttcatggtcaatgtcacagatgccatctcatccggagatgacgaggacgacgcagatggctcggaggattttgtcagtgagaacagtaacagcaagagagcaccgtactggaccaacacagaaaagatggaaaaacggctacatgcggtcccagcagccaacactgtcaagttccgctgtccagctggggggaatccaacaccaaccatgaggtggctgaaaaacgggaaggaatttaagcaggagcatcgcattggaggctataaggtacgaaaccagcattggagccttattatggaaagcgtggtcccatctgacaaaggcaattacacctgcgtggtggagaacgattacgggtccatcaatcacacgtaccacctcgacgttgttgagcgatcaccacaccggcccatccttcaagccgggctgccggcaaatgcctccaccgtggttggaggcgatgtggagtttgtctgcaaagtgtacagtgatgcccagccccatatccagtggatcaaacacgtggaaaagaatggcagtaaatacgggcccgacgggctgccctatctcaaggttctgaagcactcggggataaatagttccaatgcagaagtgctggctctgttcaatgtgactgaggcggatgctggggagtatatttgtaaggtctccaattatatagggcaggccaaccagtctgcctggctcactgtcctgccaaaacagcaagctcctgtaagggaaaaggagatgacaccttccccagactacctggaaatagccatttactgcataggggtgttctttatcgcctgcatggtggtgaccgtcatcctgtgccggatgaggaacacgaccaagaagccggacttcagcagccagccggctgtgcacaagctgaccaagcgcatccccctgcggagacaggtttctgctgagtccagctcctccatgaactccaacaccccgctggtgaggattacaactcgcctctcttcagctgcagacacccccatgctggcgggggtctccgagtacgagcttccagaagatcccaaatgggagtttccgagagataagctgacgctgggcaaacccctgggagaaggttgctttgggcaagtggtcatggctgaagcagtgggaattgacaaggagaagcccaaggaagcagtcactgtggccgtgaagatgttgaaagatgatgccactgagaaagacctttctgatctggtgtccgagatggagatgatgaagatgattgggaaacacaaaaatatcataaatctccttggagcctgtactcaggatgggccgctctatgtcatcgtcgaatacgcctcgaaaggcaaccttcgggaatacctccgcgcccggaggccacccgggatggagtattcctatgacatcagccgcgttcccgaggagcagatggccttcaaggacctggtgtcgtgcacctaccagctggcccggggcatggagtacttggcttcccagaaatgcattcatcgagatttagctgccagaaatgttttggtaacagaaaacaacgtgatgaaaatagctgactttggactggccagagatatcaacaatatagactattacaaaaagaccacaaatggccgacttccggtcaagtggatggctcccgaagcccttttcgacagagtgtacacccatcagagcgatgtctggtccttcggggtgttaatgtgggagatcttcacgttagggggctcgccctacccagggattcccgtggaggaactttttaagctgcttaaggagggacataggatggacaagccagcaaactgcaccaacgaactgtatatgatgatgagagattgctggcatgcagtgccctcacagagacccaccttcaagcagttggtagaagacttggatcgaattctcacactcacaaccaacgaggaatacttggacctcagtcagcttcttgaacagtattcacctagttaccctgacacaaggagttcttgctcttcgggagatgattctgttttctctccggaccccatgccttacgaaccctgccttcctcagtatccacatagaaacggcagtgttaaaaca

SEQ ID NO: 9 - DNA, 1200 bp, Cervus nippon
  source 1..1200: mol_type = genomic DNA
atggaggtagagggtcaggggctgtacagtaacaggcggtacccaggcaacatgggtgactggagtgccttaggcaaactccttgacaaggttcaagcctattccaccgctggagggaaggtgtggctgtccgtccttttcattttccgaatcctgctattggggacagcggttgagtcagcctggggtgatgagcagtccgcctttcgttgtaacactcaacaacctggttgtgaaaatgtctgctatgacaaatccttcccaatctctcatgtgcgcttctgggtcctgcagatcatatttgtgtctgttcccacactcttatacctggctcatgtgttctatgtgatgcgaaaggaagagaaactgaacaagaaagaggaggaactcaaagttgcccaaactgatggtgccaatgtggacatgcacttgaagcagattgaaattaagaagttcaagtatggcattgaagagcacggcaaagtgaagatgcgagggggcttgctgagaacctacatcatcagcattctcttcaagtctgtcttcgaggtggccttcttgctgatccagtggtacatctacggattcagcttgagtgccgtttacacttgcaaaagagatccctgcccgcatcaggtggactgtttcctctctcggcccacggagaaaaccatcttcatcatcttcatgctggtcgtgtcgttggtgtcgcttgccttgaacatcatcgaactcttctatgtcttcttcaagggtgttaaggatcgtgtgaagggaaagagcgatccttaccacactaccaccggcccactgagcccctccaaagactgtggatctccaaaatatgcttatttcaatggctgctcttccccaaccgctcctctctcgcccatgtctcctcccgggtacaagctagtcaccggagacagaaacaattcttcttgccgcaattacaacaaacaagcaagtgagcaaaactgggccaattacagcgcagaacaaaatcgaatggggcaggcaggcagcaccatctccaactcccacgcacagccttttgatttcccagatgaccaccagaattctaaaaaacttgatgctggccacgaactacagcctctagccattgtggaccagcggccttccagcagagccagcagtcgcgccagcagccgaccccggcctgatgacctggagatctag